European Patent Specification EP 3 922 718 B1, published December 17, 2025. Title: A Heat-resistant DNA Polymerase Mutant with High Amplification Activity. Applicant: Daan Gene Co., Ltd. Of Sun Yat-Sen University. The sequence listing filed with the application follows.

SEQUENCE LISTING (12 sequences)

SEQ ID NO: 1 - DNA, 2496 bp, Artificial sequence
  Polynucleotide
atgcgtggcatgctgccgcttttcgagcctaagggacgcgttcttcttgtggatggacatcatctggcgtaccgtacctttcatgccctgaagggcctgaccacttcgcgtggggaacccgtgcaagcagtttatggattcgccaaatcgttacttaaggctctgaaggaggatggtgatgcggtcattgttgtgttcgacgcaaaagctccctcgttccgtcacgaggcctacggcggctataaagctgggcgtgcacccacacctgaggattttccccggcaacttgctttgataaaggaattagtagacctgttaggcctggcgcggttagaagtgccgggttacgaagcagatgacgtcttggctagtttagcgaaaaaggctgaaaaagagggatatgaagtgcggatcctgaccgcggataaagatctgtatcaactgttgtccgaccgtattcacgtgcttcatccggagggctacttgataaccccggcttggctgtgggagaaatatgggctgcgtccagatcagtgggctgattatcgtgcacttacaggcgatgaatctgataatcttcccggcgtcaaggggattggtgagaaaaccgcccgtaaacttttggaggagtggggcagcttggaggcgctgttgaagaatctggatcgtttgaaacccgctatacgggaaaaaatcttggcgcacatggacgacttaaaactgtcttgggacctggcgaaagttcgtactgatttgccgctggaggtcgactttgcgaagcgtcgcgagcccgatcgtgaacgtcttcgcgcatttctggagcgtttagaatttggctccctgttgcatgagtttggtttgcttgaaagcccgaaggcacttgaggaagctccttggcctccgcctgagggcgcttttgtcggatttgtcttgagccgtaaagaaccgatgtgggcggacttactggcccttgctgctgctcgtgggggtcgcgtgcatcgcgcaccggagccatacaaagcacttcgtgaccttaaagaagcccgtggcttgttggcaaaagatttaagtgtcctggctttacgcgagggcttgggcttaccaccgggagatgatccgatgcttttggcctatctgctggacccgagcaacacgactccagagggcgttgcccgtcgttatggcggagaatggacggaggaggcgggagagcgcgcagcgttaagcgagcgtctgtttgctaatctgtggggacgcttagagggagaggagcgcctgttgtggttgtaccgtgaagtggaacggccgctgagtgcagtgttagctcacatggaagcaaccggggtgcggctggacgttgcgtatttgcgtgcgctgtcgttagaggtcgcggaggaaatagcccgtctggaggccgaagtattccgtttggctggccatcctttcaacctgaacagtcgggatcagctggaacgtgtactttttgatgaactggggctgcccgccatcggcaaaaccgaaaaaaccggcaaacgtagcacctctgcggcagtgctggaagcgttacgtgaagctcatccgattgtggagaaaattctgcaatatcgcgaattgacgaaactgaagagcacctatattgatccgctgccagacttaattcacccccgtaccggacggttgcatacccgcttcaaccagaccgcgacggcgacagggcggctgagtagcagcgatccgaacctgcaaaacattcccgtgcgtaccccgctgggtcagcgtattcgccgtgctttcattgccgaggaaggctggctgctggtcgcgctggactactcgcaaatcgaattgcgtgtgttggcccacctgtcgggcgacgaaaacttaatacgcgtgtttcaagaaggtcgtgacatacatactgaaaccgcgtcctggatgtttggagtcccacgggaggctgtcgatcctcttatgcgtcgtgccgccaaaacaattaacttcggagttctgtacggcatgtcggcacatcgtttatcacaggaactggcgattccgtatgaagaagcgcaggccttcatagaacgttatttccaatcattccccaaggtgcgggcctggattgagaagaccctggaagagggccgtcgtcgtggctatgtagagactctgttcggacgtcggcggtatgtacccgatcttgaggcccgtgtgaagtccgttcgtgaggcagcagaacgtatggcgtttaacatgccagtccagggcacagcggcggacctgatgaaattagctatggttaagctgtttccgcgtttggaagaaatgggcgctcgtatgctgttacaggttcatgacgagttagtattagaagcaccgaaggagcgtgccgaagccgtggcccggttagccaaagaggtaatggaaggcgtctacccccttgcagtcccgcttgaagtcgaagttggcataggggaagactggttatctgcgaaggaa

SEQ ID NO: 2 - protein, 832 aa, Artificial sequence [sequence omitted]

SEQ ID NO: 3 - DNA, 1269 bp, Artificial sequence
  Polynucleotide
atgcgtggcatgctgccgcttttcgagcctaagggacgcgttcttcttgtggatggacatcatctggcgtaccgtacctttcatgccctgaagggcctgaccacttcgcgtggggaacccgtgcaagcagtttatggattcgccaaatcgttacttaaggctctgaaggaggatggtgatgcggtcattgttgtgttcgacgcaaaagctccctcgttccgtcacgaggcctacggcggctataaagctgggcgtgcacccacacctgaggattttccccggcaacttgctttgataaaggaattagtagacctgttaggcctggcgcggttagaagtgccgggttacgaagcagatgacgtcttggctagtttagcgaaaaaggctgaaaaagagggatatgaagtgcggatcctgaccgcggataaagatctgtatcaactgttgtccgaccgtattcacgtgcttcatccggagggctacttgataaccccggcttggctgtgggagaaatatgggctgcgtccagatcagtgggctgattatcgtgcacttacaggcgatgaatctgataatcttcccggcgtcaaggggattggtgagaaaaccgcccgtaaacttttggaggagtggggcagcttggaggcgctgttgaagaatctggatcgtttgaaacccgctatacgggaaaaaatcttggcgcacatggacgacttaaaactgtcttgggacctggcgaaagttcgtactgatttgccgctggaggtcgactttgcgaagcgtcgcgagcccgatcgtgaacgtcttcgcgcatttctggagcgtttagaatttggctccctgttgcatgagtttggtttgcttgaaagcccgaaggcacttgaggaagctccttggcctccgcctgagggcgcttttgtcggatttgtcttgagccgtaaagaaccgatgtgggcggacttactggcccttgctgctgctcgtgggggtcgcgtgcatcgcgcaccggagccatacaaagcacttcgtgaccttaaagaagcccgtggcttgttggcaaaagatttaagtgtcctggctttacgcgagggcttgggcttaccaccgggagatgatccgatgcttttggcctatctgctggacccgagcaacacgactccagagggcgttgcccgtcgttatggcggagaatggacggaggaggcgggagagcgcgcagcgttaagcgagcgtctgtttgctaatctgtggggacgcttagagggagag

SEQ ID NO: 4 - DNA, 30 bp, Artificial sequence
  Primer
atatcatatgcgtggcatgctgccgctttt

SEQ ID NO: 5 - DNA, 30 bp, Artificial sequence
  Primer
gcatgaattccgtctcctctccctctaagc

SEQ ID NO: 6 - DNA, 1236 bp, Artificial sequence
  Polynucleotide
ggagaggagcgcctgttgtggttgtaccgtgaagtggaacggccgctgagtgcagtgttagctcacatggaagcaaccggggtgcggctggacgttgcgtatttgcgtgcgctgtcgttagaggtcgcggaggaaatagcccgtctggaggccgaagtattccgtttggctggccatcctttcaacctgaacagtcgggatcagctggaacgtgtactttttgatgaactggggctgcccgccatcggcaaaaccgaaaaaaccggcaaacgtagcacctctgcggcagtgctggaagcgttacgtgaagctcatccgattgtggagaaaattctgcaatatcgcgaattgacgaaactgaagagcacctatattgatccgctgccagacttaattcacccccgtaccggacggttgcatacccgcttcaaccagaccgcgacggcgacagggcggctgagtagcagcgatccgaacctgcaaaacattcccgtgcgtaccccgctgggtcagcgtattcgccgtgctttcattgccgaggaaggctggctgctggtcgcgctggactactcgcaaatcgaattgcgtgtgttggcccacctgtcgggcgacgaaaacttaatacgcgtgtttcaagaaggtcgtgacatacatactgaaaccgcgtcctggatgtttggagtcccacgggaggctgtcgatcctcttatgcgtcgtgccgccaaaacaattaacttcggagttctgtacggcatgtcggcacatcgtttatcacaggaactggcgattccgtatgaagaagcgcaggccttcatagaacgttatttccaatcattccccaaggtgcgggcctggattgagaagaccctggaagagggccgtcgtcgtggctatgtagagactctgttcggacgtcggcggtatgtacccgatcttgaggcccgtgtgaagtccgttcgtgaggcagcagaacgtatggcgtttaacatgccagtccagggcacagcggcggacctgatgaaattagctatggttaagctgtttccgcgtttggaagaaatgggcgctcgtatgctgttacaggttcatgacgagttagtattagaagcaccgaaggagcgtgccgaagccgtggcccggttagccaaagaggtaatggaaggcgtctacccccttgcagtcccgcttgaagtcgaagttggcataggggaagactggttatctgcgaaggaataa

SEQ ID NO: 7 - DNA, 25 bp, Artificial sequence
  Primer
ggagaggagcgcctgttgtggttgt

SEQ ID NO: 8 - DNA, 25 bp, Artificial sequence
  Primer
ttattccttcgcagataaccagtct

SEQ ID NO: 9 - DNA, 21 bp, Artificial sequence
  Primer
tacggttaaccctttgaatca

SEQ ID NO: 10 - DNA, 21 bp, Artificial sequence
  Primer
gttacctggttaaactgtact

SEQ ID NO: 11 - DNA, 38 bp, Artificial sequence
  Primer
atgcgtggcatgctgccgcttttcgagcctaagggacg

SEQ ID NO: 12 - DNA, 42 bp, Artificial sequence
  Primer
ttccttcgcagataaccagtcttcccctatgccaacttcgac